European Patent Application EP 4 261 278 A1, published October 18, 2023. Title: 一种鼠抗NDM型碳青霉烯酶杂交瘤细胞株，单克隆抗体及应用. Applicant: 天津一瑞生物科技股份有限公司. The sequence listing filed with the application follows.

SEQUENCE LISTING (20 sequences)

SEQ ID NO: 1 - protein, 16 aa, Artificial sequence
RSSQSIVHSDGNTYLD

SEQ ID NO: 2 - protein, 7 aa, Artificial sequence
KVSNRFS

SEQ ID NO: 3 - protein, 9 aa, Artificial sequence
FQISRVPFT

SEQ ID NO: 4 - protein, 10 aa, Artificial sequence
GYAFSNYLIE

SEQ ID NO: 5 - protein, 17 aa, Artificial sequence
VINPGRDDTNYNEKFKG

SEQ ID NO: 6 - protein, 19 aa, Artificial sequence
FPSILRYDSGSFSYFGLDC

SEQ ID NO: 7 - protein, 114 aa, Artificial sequence
DVLMTQTPLSLSVSLGDQASISCRSSQSIVHSDGNTYLDWYLQKPGQSPKLLIYKVSNRFSGVPDRFSGSGSGTDFTLKITRVEAEDLGVYYCFQISRVPFTFGSGTKLEIKRA

SEQ ID NO: 8 - DNA, 342 bp, Artificial sequence
  source 1..342: mol_type = other DNA
gatgttttgatgacccaaactccactctccctgtctgtcagtcttggagatcaagcctccatctcttgcagatctagtcagagcattgtacatagtgatggaaacacctatttagactggtatctgcagaaaccaggccagtctccaaaactcctaatctacaaagtttccaaccgattttctggggtcccagacaggttcagtggcagtggatcagggacagatttcacactcaagatcaccagagtggaggctgaggatctgggagtttattactgctttcaaatttcacgtgttccattcacgttcggctcggggacaaagttggaaataaaacgggct

SEQ ID NO: 9 - protein, 128 aa, Artificial sequence
SRDYGLRVELVRPGTSVKVSCKASGYAFSNYLIEWVKQRPGQGLEWIGVINPGRDDTNYNEKFKGKATLTADKSSSTAYMHLSSLTSDDSAVYFCARFPSILRYDSGSFSYFGLDCWGQGTSVTVSSA

SEQ ID NO: 10 - DNA, 384 bp, Artificial sequence
  source 1..384: mol_type = other DNA
tccagagattatggacttcgggttgagctggtaaggcctgggacttcagtgaaggtgtcctgcaaggcttctggatacgccttcagtaattacttgatagagtgggtaaagcagaggcctggacagggccttgagtggattggagtgattaatcctggaagggatgatactaactacaatgagaagttcaagggcaaggcaacactgactgcagacaaatcctccagcactgcctacatgcacctcagcagtctgacatctgatgactctgcggtctacttctgtgcaagattcccttctattcttcgctacgatagtggctctttttcttattttggtttggactgctggggtcaaggaacctcagtcaccgtctcttcagcc

SEQ ID NO: 11 - protein, 17 aa, Artificial sequence
RSSQSLFNSGNQKNYLT

SEQ ID NO: 12 - protein, 7 aa, Artificial sequence
WAVTRES

SEQ ID NO: 13 - protein, 9 aa, Artificial sequence
QNDYSYPLT

SEQ ID NO: 14 - protein, 10 aa, Artificial sequence
GYTLSDYHVK

SEQ ID NO: 15 - protein, 17 aa, Artificial sequence
DIRPQNGDIVYNQKFKD

SEQ ID NO: 16 - protein, 11 aa, Artificial sequence
HYYAYGKWFPY

SEQ ID NO: 17 - protein, 113 aa, Artificial sequence
DILMTQSPSSLTVTAGEKVTLSCRSSQSLFNSGNQKNYLTWHQQKPGQSPKLLIYWAVTRESGVPDRFTGSGSGTDFTLTISSVQAEDLAIYYCQNDYSYPLTFGAGTKLELK

SEQ ID NO: 18 - DNA, 339 bp, Artificial sequence
  source 1..339: mol_type = other DNA
gacattctgatgacacagtctccctcctccctgactgtgacagcaggcgagaaggtcactttgagctgcaggtccagtcagagtctgtttaacagtggaaatcaaaagaactacttgacctggcaccagcagaaaccagggcagtctcctaaattgttgatctactgggcagtcactagggaatctggggtccctgatcgcttcacaggcagtggatctggaacagatttcactctcaccatcagcagtgtgcaggctgaagacctggcaatttattactgtcagaatgattatagttatccgctcacgttcggtgctgggaccaaactggaactgaaa

SEQ ID NO: 19 - protein, 118 aa, Artificial sequence
VQLHESGPELVKPGASVKLSCTASGYTLSDYHVKWVKQNHGQSLEWIGDIRPQNGDIVYNQKFKDKATLTVDKSSTTAYIRLSSLTSEDSAVYYCAFHYYAYGKWFPYWGQGTLVTVS

SEQ ID NO: 20 - DNA, 354 bp, Artificial sequence
  source 1..354: mol_type = other DNA
gtgcagcttcacgagtcaggacctgagctggtgaagcctggggcttcagtgaaactgtcctgcacggcttccggatacaccctcagtgactaccacgtaaaatgggtgaaacagaaccatggacagagccttgagtggattggagatattaggcctcagaatggtgatattgtttacaaccagaagttcaaggacaaggccacattgactgtagacaaatcctccacaacagcctacatacgactcagcagcctgacatctgaggactctgcagtctattactgtgcattccattattacgcctacgggaagtggtttccttattggggccaagggactctggtcaccgtctcc